European Patent Application EP 4 755 403 A1, published June 10, 2026. Title: 抗PSMA抗体药物偶联物及其医药用途. Applicant: 江苏恒瑞医药股份有限公司. Application WO. The sequence listing filed with the application follows.

SEQUENCE LISTING (32 sequences)

SEQ ID NO: 1 - protein, 750 aa, Homo sapiens
MWNLLHETDSAVATARRPRWLCAGALVLAGGFFLLGFLFGWFIKSSNEATNITPKHNMKAFLDELKAENIKKFLYNFTQIPHLAGTEQNFQLAKQIQSQWKEFGLDSVELAHYDVLLSYPNKTHPNYISIINEDGNEIFNTSLFEPPPPGYENVSDIVPPFSAFSPQGMPEGDLVYVNYARTEDFFKLERDMKINCSGKIVIARYGKVFRGNKVKNAQLAGAKGVILYSDPADYFAPGVKSYPDGWNLPGGGVQRGNILNLNGAGDPLTPGYPANEYAYRRGIAEAVGLPSIPVHPIGYYDAQKLLEKMGGSAPPDSSWRGSLKVPYNVGPGFTGNFSTQKVKMHIHSTNEVTRIYNVIGTLRGAVEPDRYVILGGHRDSWVFGGIDPQSGAAVVHEIVRSFGTLKKEGWRPRRTILFASWDAEEFGLLGSTEWAEENSRLLQERGVAYINADSSIEGNYTLRVDCTPLMYSLVHNLTKELKSPDEGFEGKSLYESWTKKSPSPEFSGMPRISKLGSGNDFEVFFQRLGIASGRARYTKNWETNKFSGYPLYHSVYETYELVEKFYDPMFKYHLTVAQVRGGMVFELANSIVLPFDCRDYAVVLRKYADKIYSISMKHPQEMKTYSVSFDSLFSAVKNFTEIASKFSERLQDFDKSNPIVLRMMNDQLMFLERAFIDPLGLPDRPFYRHVIYAPSSHNKYAGESFPGIYDALFDIESKVDPSKAWGEVKRQIYVAAFTVQAAAETLSEVA

SEQ ID NO: 2 - protein, 750 aa, Macaca fascicularis
MWNLLHETDSAVATARRPRWLCAGALVLAGGFFLLGFLFGWFIKSSSEATNITPKHNMKAFLDELKAENIKKFLHNFTQIPHLAGTEQNFQLAKQIQSQWKEFGLDSVELTHYDVLLSYPNKTHPNYISIINEDGNEIFNTSLFEPPPAGYENVSDIVPPFSAFSPQGMPEGDLVYVNYARTEDFFKLERDMKINCSGKIVIARYGKVFRGNKVKNAQLAGATGVILYSDPADYFAPGVKSYPDGWNLPGGGVQRGNILNLNGAGDPLTPGYPANEYAYRRGIAEAVGLPSIPVHPIGYYDAQKLLEKMGGSASPDSSWRGSLKVPYNVGPGFTGNFSTQKVKMHIHSTSEVTRIYNVIGTLRGAVEPDRYVILGGHRDSWVFGGIDPQSGAAVVHEIVRSFGTLKKEGWRPRRTILFASWDAEEFGLLGSTEWAEENSRLLQERGVAYINADSSIEGNYTLRVDCTPLMYSLVYNLTKELESPDEGFEGKSLYESWTKKSPSPEFSGMPRISKLGSGNDFEVFFQRLGIASGRARYTKNWETNKFSSYPLYHSVYETYELVEKFYDPMFKYHLTVAQVRGGMVFELANSVVLPFDCRDYAVVLRKYADKIYNISMKHPQEMKTYSVSFDSLFSAVKNFTEIASKFSERLRDFDKSNPILLRMMNDQLMFLERAFIDPLGLPDRPFYRHVIYAPSSHNKYAGESFPGIYDALFDIESKVDPSQAWGEVKRQISIATFTVQAAAETLSEVA

SEQ ID NO: 3 - protein, 119 aa, synthetic construct
  source 1..119: note = HV
EVKLVESEGGLVQPGSSMKLSCTASGFTFSDYYMAWVRQVPERGLEWVANINYDGSSTYYLDSLKSRFIISRDNAKNILYLQMSSLKSEDTATYYCARGGDYWDAMDYWGQGTSVTVSS

SEQ ID NO: 4 - protein, 107 aa, synthetic construct
  source 1..107: note = LV
DIQMTQTTSSLSASLGDRVTISCRASQDISKYLNWYQQKPDGTVKLLIYYTSSLHSGVPSRFSGSGSGTDYSLTISNLEQEDIATYFCQQGNRLPRTFGGGTKLEIK

SEQ ID NO: 5 - protein, 5 aa, synthetic construct
  source 1..5: note = CDR
DYYMA

SEQ ID NO: 6 - protein, 17 aa, synthetic construct
  source 1..17: note = CDR
NINYDGSSTYYLDSLKS

SEQ ID NO: 7 - protein, 10 aa, synthetic construct
  source 1..10: note = CDR
GGDYWDAMDY

SEQ ID NO: 8 - protein, 11 aa, synthetic construct
  source 1..11: note = CDR
RASQDISKYLN

SEQ ID NO: 9 - protein, 7 aa, synthetic construct
  source 1..7: note = CDR
YTSSLHS

SEQ ID NO: 10 - protein, 9 aa, synthetic construct
  source 1..9: note = CDR
QQGNRLPRT

SEQ ID NO: 11 - protein, 119 aa, synthetic construct
  source 1..119: note = VH
EVQLVESGGGLVQPGGSLRLSCAASGFTFSDYYMAWVRQAPGKGLEWVANINYDGSSTYYLDSLKSRFTISRDNAKNSLYLQMNSLRAEDTAVYYCARGGDYWDAMDYWGQGTTVTVSS

SEQ ID NO: 12 - protein, 119 aa, synthetic construct
  source 1..119: note = VH
EVKLVESGGGLVQPGGSLRLSCAASGFTFSDYYMAWVRQAPGKGLEWVANINYDGSSTYYLDSLKSRFTISRDNAKNSLYLQMNSLRAEDTAVYYCARGGDYWDAMDYWGQGTTVTVSS

SEQ ID NO: 13 - protein, 107 aa, synthetic construct
  source 1..107: note = VL
DIQMTQSPSSLSASVGDRVTITCRASQDISKYLNWYQQKPGKAPKLLIYYTSSLHSGVPSRFSGSGSGTDFTLTISSLQPEDFATYYCQQGNRLPRTFGGGTKVEIK

SEQ ID NO: 14 - protein, 107 aa, synthetic construct
  source 1..107: note = VL
DIQMTQSPSSLSASVGDRVTITCRASQDISKYLNWYQQKPGKAPKLLIYYTSSLHSGVPSRFSGSGSGTDYTLTISSLQPEDFATYYCQQGNRLPRTFGGGTKVEIK

SEQ ID NO: 15 - protein, 330 aa, Homo sapiens [sequence omitted]

SEQ ID NO: 16 - protein, 330 aa, synthetic construct
  source 1..330: note = constant region
ASTKGPSVFPLAPSSKSTSGGTAALGCLVKDYFPEPVTVSWNSGALTSGVHTFPAVLQSSGLYSLSSVVTVPSSSLGTQTYICNVNHKPSNTKVDKKVEPKSSDKTHTCPPCPAPELLGGPSVFLFPPKPKDTLMISRTPEVTCVVVDVSHEDPEVKFNWYVDGVEVHNAKTKPREEQYNSTYRVVSVLTVLHQDWLNGKEYKCKVSNKALPAPIEKTISKAKGQPREPQVYTLPPSRDELTKNQVSLTCLVKGFYPSDIAVEWESNGQPENNYKTTPPVLDSDGSFFLYSKLTVDKSRWQQGNVFSCSVMHEALHNHYTQKSLSLSPGK

SEQ ID NO: 17 - protein, 107 aa, Homo sapiens [sequence omitted]

SEQ ID NO: 18 - protein, 107 aa, Homo sapiens
RTVAAPSVFIFPPSDEQLKSGTASVVCLLNNFYPREAKVQWKVDNALQSGNSQESVTEQDSKDSTYSLSSTLTLSKADYEKHKVYACEVTHQGLSSPVTKSFNRGES

SEQ ID NO: 19 - protein, 449 aa, synthetic construct
  source 1..449: note = HC
EVKLVESGGGLVQPGGSLRLSCAASGFTFSDYYMAWVRQAPGKGLEWVANINYDGSSTYYLDSLKSRFTISRDNAKNSLYLQMNSLRAEDTAVYYCARGGDYWDAMDYWGQGTTVTVSSASTKGPSVFPLAPSSKSTSGGTAALGCLVKDYFPEPVTVSWNSGALTSGVHTFPAVLQSSGLYSLSSVVTVPSSSLGTQTYICNVNHKPSNTKVDKKVEPKSCDKTHTCPPCPAPELLGGPSVFLFPPKPKDTLMISRTPEVTCVVVDVSHEDPEVKFNWYVDGVEVHNAKTKPREEQYNSTYRVVSVLTVLHQDWLNGKEYKCKVSNKALPAPIEKTISKAKGQPREPQVYTLPPSRDELTKNQVSLTCLVKGFYPSDIAVEWESNGQPENNYKTTPPVLDSDGSFFLYSKLTVDKSRWQQGNVFSCSVMHEALHNHYTQKSLSLSPGK

SEQ ID NO: 20 - protein, 214 aa, synthetic construct
  source 1..214: note = LC
DIQMTQSPSSLSASVGDRVTITCRASQDISKYLNWYQQKPGKAPKLLIYYTSSLHSGVPSRFSGSGSGTDYTLTISSLQPEDFATYYCQQGNRLPRTFGGGTKVEIKRTVAAPSVFIFPPSDEQLKSGTASVVCLLNNFYPREAKVQWKVDNALQSGNSQESVTEQDSKDSTYSLSSTLTLSKADYEKHKVYACEVTHQGLSSPVTKSFNRGEC

SEQ ID NO: 21 - protein, 453 aa, synthetic construct
  source 1..453: note = HC
QVQLVESGGGVVQPGRSLRLSCAASGFAFSRYGMHWVRQAPGKGLEWVAVIWYDGSNKYYADSVKGRFTISRDNSKNTQYLQMNSLRAEDTAVYYCARGGDFLYYYYYGMDVWGQGTTVTVSSASTKGPSVFPLAPSSKSTSGGTAALGCLVKDYFPEPVTVSWNSGALTSGVHTFPAVLQSSGLYSLSSVVTVPSSSLGTQTYICNVNHKPSNTKVDKKVEPKSCDKTHTCPPCPAPELLGGPSVFLFPPKPKDTLMISRTPEVTCVVVDVSHEDPEVKFNWYVDGVEVHNAKTKPREEQYNSTYRVVSVLTVLHQDWLNGKEYKCKVSNKALPAPIEKTISKAKGQPREPQVYTLPPSRDELTKNQVSLTCLVKGFYPSDIAVEWESNGQPENNYKTTPPVLDSDGSFFLYSKLTVDKSRWQQGNVFSCSVMHEALHNHYTQKSLSLSPGK

SEQ ID NO: 22 - protein, 214 aa, synthetic construct
  source 1..214: note = LC
DIQMTQSPSSLSASVGDRVTITCRASQGISNYLAWYQQKTGKVPKFLIYEASTLQSGVPSRFSGGGSGTDFTLTISSLQPEDVATYYCQNYNSAPFTFGPGTKVDIKRTVAAPSVFIFPPSDEQLKSGTASVVCLLNNFYPREAKVQWKVDNALQSGNSQESVTEQDSKDSTYSLSSTLTLSKADYEKHKVYACEVTHQGLSSPVTKSFNRGEC

SEQ ID NO: 23 - protein, 448 aa, synthetic construct
  source 1..448: note = HC
QVQLVQSGAEVKKPGASVKVSCKASGYTFTNSWIGWFRQAPGQGLEWIGDIYPGGGYTNYNEIFKGKATMTADTSTNTAYMELSSLRSEDTAVYYCSRGIPGYAMDYWGQGTLVTVSSASTKGPSVFPLAPSSKSTSGGTAALGCLVKDYFPEPVTVSWNSGALTSGVHTFPAVLQSSGLYSLSSVVTVPSSSLGTQTYICNVNHKPSNTKVDKKVEPKSCDKTHTCPPCPAPELLGGPSVFLFPPKPKDTLMISRTPEVTCVVVDVSHEDPEVKFNWYVDGVEVHNAKTKPREEQYNSTYRVVSVLTVLHQDWLNGKEYKCKVSNKALPAPIEKTISKAKGQPREPQVYTLPPSRDELTKNQVSLTCLVKGFYPSDIAVEWESNGQPENNYKTTPPVLDSDGSFFLYSKLTVDKSRWQQGNVFSCSVMHEALHNHYTQKSLSLSPGK

SEQ ID NO: 24 - protein, 220 aa, synthetic construct
  source 1..220: note = LC
DIQMTQSPSSLSASVGDRVTMSCKSSQSLLNSGDQKNYLTWYQQKPGKAPKLLIYWASTGESGVPSRFSGSGSGTDFTFTISSLQPEDIATYYCQNDYSYPWTFGQGTKVEIKRTVAAPSVFIFPPSDEQLKSGTASVVCLLNNFYPREAKVQWKVDNALQSGNSQESVTEQDSKDSTYSLSSTLTLSKADYEKHKVYACEVTHQGLSSPVTKSFNRGEC

SEQ ID NO: 25 - protein, 4 aa, synthetic construct
  source 1..4: note = linker
GGFG

SEQ ID NO: 26 - protein, 8 aa, synthetic construct
  source 1..8: note = CDR
GFTFSDYY

SEQ ID NO: 27 - protein, 8 aa, synthetic construct
  source 1..8: note = CDR
INYDGSST

SEQ ID NO: 28 - protein, 12 aa, synthetic construct
  source 1..12: note = CDR
ARGGDYWDAMDY

SEQ ID NO: 29 - protein, 6 aa, synthetic construct
  source 1..6: note = CDR
QDISKY

SEQ ID NO: 30 - skipped

SEQ ID NO: 31 - protein, 7 aa, synthetic construct
  source 1..7: note = CDR
GFTFSDY

SEQ ID NO: 32 - protein, 6 aa, synthetic construct
  source 1..6: note = CDR
NYDGSS